European Patent Specification EP 3 454 884 B1, published July 12, 2023. Title: AGENTS THAT ACTIVATE CD47 AND THEIR USE IN THE TREATMENT OF INFLAMMATION. Applicant: Université Pierre-et-Marie-Curie Centre National de la Recherche Scientifique Institut National de la Santé et de la Recherche Médicale SENNLAUB Florian HOUSSET Michael GUILLONEAU Xavier SAHEL José-Alain KAROYAN Philippe. The sequence listing filed with the application follows.

SEQUENCE LISTING (14 sequences)

SEQ ID NO: 1 - protein, 10 aa, Artificial Sequence
  4N1K peptide
KRFYVVMWKK

SEQ ID NO: 2 - protein, 8 aa, Artificial Sequence
  Peptide linker
GGGKGGGG

SEQ ID NO: 3 - protein, 8 aa, Artificial Sequence
  Peptide linker
GGGNGSGG

SEQ ID NO: 4 - protein, 8 aa, Artificial Sequence
  Peptide linker
GGGCGGGG

SEQ ID NO: 5 - protein, 4 aa, Artificial Sequence
  Peptide linker
GPNG

SEQ ID NO: 6 - protein, 8 aa, Artificial Sequence
  Peptide linker
GGGGGGGG

SEQ ID NO: 7 - protein, 28 aa, Artificial Sequence
  4N1K dimer
KRFYVVMWKKGGGGGGGGKRFYVVMWKK

SEQ ID NO: 8 - protein, 369 aa, Homo sapiens
  TSP-1 C-terminal
MACPGFLWALVISTCLEFSMADYKDDDDKALADCCPLEHNPDQLDSDSDRIGDTCDNNQDIDEDGHQNNLDNCPYVPNANQADHDKDGKGDACDHDDDNDGIPDDKDNCRLVPNPDQKDSDGDGRGDACKDDFDHDSVPDIDDICPENVDISETDFRRFQMIPLDPKGTSQNDPNWVVRHQGKELVQTVNCDPGLAVGYDEFNAVDFSGTFFINTERDDDYAGFVFGYQSSSRFYVVMWKQVTQSYWDTNPTRAQGYSGLSVKVVNSTTGPGEHLRNALWHTGNTPGQVRTLWHDPRHIGWKDFTAYRWRLSHRPKTGFIRVVMYEGKKIMADSGPIYDKTYAGGRLGLFVFSQEMVFFSDLKYECRDP

SEQ ID NO: 9 - protein, 365 aa, Artificial Sequence
  Modified TSP-1 C-terminal
MACPGFLWALVISTCLEFSMADYKDDDDKALCDNCPLEHNPDQLDSDSDRIGDTCDNNQDIDEDGHQNNLDNCPYVPNANQADHDKDGKGDACDHDDDNDGIPDDKDNCRLVPNPDQKDSDGDGRGDACKDDFDHDSVPDIDDICPENVDISETDFRRFQMIPLDPKGTSQNDPNWVVRHQGKELVQTVNCDPGLAVGYDEFNAVDFSGTFFINTERDDDYAGFVFGYQSSSRFYVVMWKQQSYWDTNPTRAQGYSGLSVKVVNSTTGPGEHLRNALWHTGNTPGRTLWHDPRHIGWKDFTAYRWRLSHRPKTGFIRVVMYEGKKIMADSGPIYDKTYAGGRLGLFVFSQEMVFFSDLKYECRDP

SEQ ID NO: 10 - protein, 365 aa, Artificial Sequence
  Modified TSP-1 C-terminal
MACPGFLWALVISTCLEFSMADYKDDDDKALADNCPLEHNPDQLDSDSDRIGDTCDNNQDIDEDGHQNNLDNCPYVPNANQADHDKDGKGDACDHDDDNDGIPDDKDNCRLVPNPDQKDSDGDGRGDACKDDFDHDSVPDIDDICPENVDISETDFRRFQMIPLDPKGTSQNDPNWVVRHQGKELVQTVNSDPGLAVGYDEFNAVDFSGTFFINTERDDDYAGFVFGYQSSSRFYVVMWKQQSYWDTNPTRAQGYSGLSVKVVKSTTGPGEHLRNALWHTGNTPGRTLWHDPRHIGWKDFTAYRWRLSHRPKTGFIRVVMYEGKKIMADSGPIYDKTYAGGRLGLFVFSQEMVFFSDLKYECRDP

SEQ ID NO: 11 - protein, 369 aa, Artificial Sequence
  Modified TSP-1 C-terminal
MACPGFLWALVISTCLEFSMADYKDDDDKALCDNCPLEHNPDQLDSDSDRIGDTCDNNQDIDEDGHQNNLDNCPYVPNANQADHDKDGKGDACDHDDDNDGIPDDKDNCRLVPNPDQKDSDGDGRGDACKDDFDHDSVPDIDDICPENVDISETDFRRFQMIPLDPKGTSQNDPNWVVRHQGKELVQTVNCDPGLAVGYDEFNAVDFSGTFFINTERDDDYAGFVFGYQSSSRFYVVMWKQNTQSYWDTNPTRAQGYSGLSVKVVNSTTGPGEHLRNALWHTGNTPGQNRTLWHDPRHIGWKDFTAYRWRLSHRPKTGFIRVVMYEGKKIMADSGPIYDKTYAGGRLGLFVFSQEMVFFSDLKYECRDP

SEQ ID NO: 12 - protein, 369 aa, Artificial Sequence
  Modified TSP-1 C-terminal
MACPGFLWALVISTCLEFSMADYKDDDDKALADNCPLEHNPDQLDSDSDRIGDTCDNNQDIDEDGHQNNLDNCPYVPNANQADHDKDGKGDACDHDDDNDGIPDDKDNCRLVPNPDQKDSDGDGRGDACKDDFDHDSVPDIDDICPENVDISETDFRRFQMIPLDPKGTSQNDPNWVVRHQGKELVQTVNSDPGLAVGYDEFNAVDFSGTFFINTERDDDYAGFVFGYQSSSRFYVVMWKQNTQSYWDTNPTRAQGYSGLSVKVVKSTTGPGEHLRNALWHTGNTPGQNRTLWHDPRHIGWKDFTAYRWRLSHRPKTGFIRVVMYEGKKIMADSGPIYDKTYAGGRLGLFVFSQEMVFFSDLKYECRDP

SEQ ID NO: 13 - protein, 1168 aa, Artificial Sequence
  HTRA1-resistant modified TSP1
LAWGLGVLFLMHVCGTNRIPESGGDNSVFDIFELTGAARKGSGRRLVKGPDPSSPAFRIEDANLIPPVPDDKFQDLVDAVRAEKGFLLLASLRQMKKTRGTLLALERKDHSGQVFSVVSNGKAGTLDLSLTVQGKQHVVSVEEALLATGQWKSITLFVQEDRAQLYIDCEKMENAELDVPIQSVFTRDLASKSRMYVAKGSARESHFRGLLQNVHLVFENSVEDILSKKGCQQGTSVLLTLDNNVVNGSSPAIRTNYIGHKTKDLQAICGISCDELSSMVLELRGLRTIVTTLQDSIRKVTEENKELANELRRPPLCYHNGVQYRNNEEWTVDSCTECHCQNSVTICKKVSCPIMPCSNATVPDGECCPRCWPSDSADDGWSPWSEWTSCSTSCGNGIQQRGRSCDSLNNRCLGPSIQTRACSLSKCDTRIRQDGGWSHWSPWSSCSVTCGDGVITRIRLCNSPSPQMNGKPCEGEARETKACKKDACPINGGWGPWSPWDICSVTCGGGVQKRSRLCNNPTPQFGGKDCVGDVTENQICNKQDCPIDGCLSNPCFAGVKCTSYPDGSWKCGACPPGYSGNGIQCTDVDECKEVPDACFNHNGEHRCENTDPGYNCLPCPPRYRGNQPVGVGLEAAKTEKQVCEPENPCKDGTHDCNKNAKCNYLGHYSDPMYRCECKPGYAGNGIICGEDTDLDGWPNENLVCVANATYHCKKDNCPNLPNSGQEDYDKDGIGDACDDDDDNDKIPDDRDNCPFHYNPAQYDYDRDDVGDRCDNCPYNHNPDQADTDNNGEGDACAADIDGDGILNERDNCQYVYNVDQRDTDMDGVGDQCDNCPLEHNPDQLDSDSDRIGDTCDNNQDIDEDGHQNNLDNCPYVPNANQADHDKDGKGDACDHDDDNDGIPDDKDNCRLVPNPDQKDSDGDGRGDACKDDFDHDSVPDIDDICPENVDISETDFRRFQMIPLDPKGTSQNDPNWVVRHQGKELVQTVNCDPGLAVGYDEFNAVDFSGTFFINTERDDDYAGFVFGYQSSSRFYVVMWKQVTQTYWEDQPTRAYGYSGVSLKVVNSTTGTGEHLRNALWHTGNTPGQVRTLWHDPRNIGWKDYTAYRWHLTHRPKTGYIRVVMYEGKKIMADSGPIYDKTYAGGRLGLFVFSQEMVFFSDLKYECRD

SEQ ID NO: 14 - protein, 1171 aa, Artificial Sequence
  HTRA1-resistant derived TSP2
MVWRLVLLALWVWPSTQAGHQDKDTTFDLFSISNINRKTIGAKQFRGPDPGVPAYRFVRFDYIPPVNADDLSKITKIMRQKEGFFLTAQLKQDGKSRGTLLALEGPGLSQRQFEIVSNGPADTLDLTYWIDGTRHVVSLEDVGLADSQWKNVTVQVAGETYSLHVGCDLIDSFALDEPFYEHLQAEKSRMYVAKGSARESHFRGLLQNVHLVFENSVEDILSKKGCQQGQGAEINAISENTETLRLGPHVTTEYVGPSSERRPEVCERSCEELGNMVQELSGLHVLVNQLSENLKRVSNDNQFLWELIGGPPKTRNMSACWQDGRFFAENETWVVDSCTTCTCKKFKTICHQITCPPATCASPSFVEGECCPSCLHSVDGEEGWSPWAEWTQCSVTCGSGTQQRGRSCDVTSNTCLGPSIQTRACSLSKCDTRIRQDGGWSHWSPWSSCSVTCGVGNITRIRLCNSPVPQMGGKNCKGSGRETKACQGAPCPIDGRWSPWSPWSACTVTCAGGIRERTRVCNSPEPQYGGKACVGDVQERQMCNKRSCPVDGCLSNPCFPGAQCSSFPDGSWSCGSCPVGFLGNGTHCEDLDECALVPDICFSTSKVPRCVNTQPGFHCLPCPPRYRGNQPVGVGLEAAKTEKQVCEPENPCKDKTHNCHKHAECIYLGHFSDPMYKCECQTGYAGDGLICGEDSDLDGWPNLNLVCATNATYHCIKDNCPHLPNSGQEDFDKDGIGDACDDDDDNDGVTDEKDNCQLLFNPRQADYDKDEVGDRCDNCPYVHNPAQIDTDNNGEGDACSVDIDGDDVFNERDNCPYVYNTDQRDTDGDGVGDHCDNCPLVHNPDQTDVDNDLVGDQCDNNEDIDDDGHQNNQDNCPYISNANQADHDRDGQGDACDPDDDNDGVPDDRDNCRLVFNPDQEDLDGDGRGDICKDDFDNDNIPDIDDVCPENNAISETDFRNFQMVPLDPKGTTQIDPNWVIRHQGKELVQTANSDPGIAVGFDEFGSVDFSGTFYVNTDRDDDYAGFVFGYQSSSRFYVVMWKQVTQTYWEDQPTRAYGYSGVSLKVVNSTTGTGEHLRNALWHTGNTPGQVRTLWHDPRNIGWKDYTAYRWHLTHRPKTGFIRVVMYEGKKIMADSGPIYDKTYAGGRLGLFVFSQEMVFFSDLKYECRD